European Patent Application EP 4 151 742 A1, published March 22, 2023. Title: FRUCTOSAMINE DEGLYCASE VECTOR, TRANSGENIC CELL LINE AND GENETIC ENGINEERING BACTERIA EXPRESSING FRUCTOSAMINE DEGLYCASE, AND USE OF FRUCTOSAMINE DEGLYCASE. Applicant: Wuhan Baianhuiji Biotechnology Co., Ltd. The sequence listing filed with the application follows.

SEQUENCE LISTING (8 sequences)

SEQ ID NO: 1 - protein, 328 aa, Artificial Sequence
  amino acid sequence of the fructosamine desugarase
MSQATAKVNREVQAFLQDLKGKTIDHVFFVACGGSSAIMYPSKYVFDRESKSINSDLYSANEFIQRNPVQLGEKSLVILCSHSGNTPETVKAAAFARGKGALTIAMTFKPESPLAQEAQYVAQYDWGDEALAINTNYGVLYQIVFGTLQVLENNTKFQQAIEGLDQLQAVYEKALKQEADNAKQFAKAHEKESIIYTMASGANYGVAYSYSICILMEMQWIHSHAIHAGEYFHGPFEIIDESVPFIILLGLDETRPLEERALTFSKKYGKKLTVLDAASYDFTAIDDSVKGYLAPLVLNRVLRSYADELAEERNHPLSHRRYMWKVEY

SEQ ID NO: 2 - DNA, 1082 bp, Artificial Sequence
  nucleotide sequence of a gene encoding fructosamine deglycase
ttatataacattatagtctaatgcataatggttcttcattttcagatcaatactcaactttccacatgtatcttctatgagataaaggatgatttctctcctctgccagctcgtctgcatagcttctcagcacacgattgagaacgagcggagcaagatagcctttaactgaatcgtcaattgcagtgaagtcgtaagatgcagcatcaagcacagtgagctttttgccatactttttcgagaaggtaagcgcccgctcttcaagaggtcttgtttcatctaaaccgagcaggatgataaacggcacggattcatcaataatttcaaacggtccgtgaaaatattctccggcatgaatggcgtgggaatgaatccattgcatttccatgagaatgcagatgctgtaggagtaagcgacaccgtagtttgcaccgcttgccatggtataaataatactttctttttcatgggcttttgcaaattgcttggcgttgtcagcttcctgcttaagggctttttcatatacagcctgcaattgatctaagccttcaattgcttgttggaatttcgtattgttttctaatacttgcagggttccaaaaacgatttgatacaaaacgccatagtttgtattgatcgcaagcgcctcatcaccccaatcgtactgggcaacatattgcgcttcctgcgctaaaggagactccggtttaaacgtcatcgcaatcgtaagtgcacccttgccccttgcaaacgcagcagctttgactgtctccggggtatttcccgaatgcgagcacaaaataacaagagacttttcaccaagctgaacagggttgcgctgaataaattcgttggcgctgtagaggtcggagtttattgattttgactctctgtcaaacacatacttactcggatacataatggcagaagaccctccgcatgcgacaaagaatacatgatcaatggttttccctttcaaatcctgcaagaaagcttgaacctcacgatttacttttgctgtggcctgactcaaatccttcactccccgtttttattatataacgttatataacattatatat

SEQ ID NO: 3 - protein, 331 aa, Artificial Sequence
  amino acid sequence of the fructokinase
MITNCRRPCIANPVVRLYAIDIEKNKESTVRIGIDLGGTKTEVIALGDAGEQLYRHRLPTPRDDYRQTIETIATLVDMAEQATGQRGTVGMGIPGSISPYTGVVKNANSTWLNGQPFDKDLSARLQREVRLANDANCLAVSEAVDGAAAGAQTVFAVIIGTGCGAGVAFNGRAHIGGNGTAGEWGHNPLPWMDEDELRYREEVPCYCGKQGCIETFISGTGFAMDYRRLSGHALKGSEIIRLVEESDPVAELALRRYELRLAKSLAHVVNILDPDVIVLGGGMSNVDRLYQTVGQLIKQFVFGGECETPVRKAKHGDSSGVRGAAWLWPQE

SEQ ID NO: 4 - DNA, 993 bp, Artificial Sequence
  nucleotide sequence of the fructokinase
ctcttgtggccataaccacgcagcgccgcgtacgccgctggaatcaccgtgcttcgccttacgcaccggcgtttcacattcgccgccgaagacaaattgtttaatcaactgcccaaccgtttgatataaacggtctacattgctcatcccgccccccaggacaatcacatccggatcgagaatattcacgacatgtgccagcgattttgccagccgcagctcgtagcgacgcaatgccagttccgctaccggatcgctttcttcaaccaggcggataatttcactgcctttcagcgcatgtccgctcaaacgacgataatccatcgcgaatcccgtgcccgaaataaaggtttcaatacaaccttgtttaccgcaataacaagggacttcctcgcgataacgcagttcgtcttcgtccatccacggtagcggattgtgtccccactcacctgccgtgccattgccgccgatatgcgcccgcccattgaatgccacgcccgcgccgcatcccgtgccgataatcacggcaaataccgtctgcgctcccgctgccgcgccatctactgcttctgaaaccgccagacagttagcgtcatttgccagccgcacttcccgctgcaacctcgcgcttaagtctttatcgaatggctgaccgttgagccaggttgaattggcattcttcaccacaccggtgtaaggcgaaattgagccaggaatgcccatacctaccgttccgcgctgccccgtcgcctgctccgccatatcaaccaacgtggcgatcgtttcaatagtctgccggtaatcatcacgcggcgtgggcagacgatggcggtacaactgctcccctgcatcgcccagtgcaatcacttcagttttggtgccgcctaaatcgatacctatacgcacggtactctccttatttttttcaatatcaatagcgtagagacggacaaccggattggcaatgcaaggccgccgacaattcgttatcat

SEQ ID NO: 5 - DNA, 31 bp, Artificial Sequence
  Forward primer of fructosamine deglycase
tacgtaaatatattgtaatatcagattacgt

SEQ ID NO: 6 - DNA, 34 bp, Artificial Sequence
  Reverse primer of fructosamine deglycase
gcggccgcgttatataacattatagtctaatgca

SEQ ID NO: 7 - DNA, 31 bp, Artificial Sequence
  Forward primer of fructokinase
tacgtagagaacaccggtattggtgcgtcgc

SEQ ID NO: 8 - DNA, 34 bp, Artificial Sequence
  Reverse primer of fructokinase
gcggccgcgctcttgtggccataaccacgcagcg